European Patent Application EP 4 410 373 A2, published August 7, 2024. Title: Nucleic acids for simultaneous inhibition of mTOR gene and STAT3 gene. Applicant: Curigene Co., Ltd. The sequence listing filed with the application follows.

SEQUENCE LISTING (25 sequences)

SEQ ID NO: 1 - RNA, 21 nt, synthetic construct
  modified_base 4: mod_base = OTHER; note = thymine
  modified_base 6: mod_base = OTHER; note = thymine
  modified_base 11: mod_base = OTHER; note = thymine
  modified_base 17: mod_base = OTHER; note = thymine
  modified_base 21: mod_base = OTHER; note = thymine
  misc_feature 1..21: note = antisense_mTOR of set 1
  source 1..21: mol_type = other RNA
gactgtggcatccacctgcat

SEQ ID NO: 2 - RNA, 21 nt, synthetic construct
  modified_base 2: mod_base = OTHER; note = thymine
  modified_base 6: mod_base = OTHER; note = thymine
  modified_base 14: mod_base = OTHER; note = thymine
  modified_base 20: mod_base = OTHER; note = thymine
  misc_feature 1..21: note = antisense_STAT3 of set 1
  source 1..21: mol_type = other RNA
ctgactccgcggatggacgta

SEQ ID NO: 3 - RNA, 20 nt, synthetic construct
  modified_base 4: mod_base = OTHER; note = thymine
  modified_base 6: mod_base = OTHER; note = thymine
  modified_base 11: mod_base = OTHER; note = thymine
  modified_base 17: mod_base = OTHER; note = thymine
  misc_feature 1..20: note = antisense_mTOR of set 2
  source 1..20: mol_type = other RNA
gactgtggcatccacctgca

SEQ ID NO: 4 - RNA, 20 nt, synthetic construct
  modified_base 2: mod_base = OTHER; note = thymine
  modified_base 6: mod_base = OTHER; note = thymine
  modified_base 14: mod_base = OTHER; note = thymine
  modified_base 20: mod_base = OTHER; note = thymine
  misc_feature 1..20: note = antisense_STAT3 of set 2
  source 1..20: mol_type = other RNA
ctgactccgcggatggacgt

SEQ ID NO: 5 - RNA, 19 nt, synthetic construct
  modified_base 4: mod_base = OTHER; note = thymine
  modified_base 6: mod_base = OTHER; note = thymine
  modified_base 11: mod_base = OTHER; note = thymine
  modified_base 17: mod_base = OTHER; note = thymine
  misc_feature 1..19: note = antisense_mTOR of set 3
  source 1..19: mol_type = other RNA
gactgtggcatccacctgc

SEQ ID NO: 6 - RNA, 19 nt, synthetic construct
  modified_base 2: mod_base = OTHER; note = thymine
  modified_base 6: mod_base = OTHER; note = thymine
  modified_base 14: mod_base = OTHER; note = thymine
  misc_feature 1..19: note = antisense_STAT3 of set 3
  source 1..19: mol_type = other RNA
ctgactccgcggatggacg

SEQ ID NO: 7 - RNA, 18 nt, synthetic construct
  modified_base 4: mod_base = OTHER; note = thymine
  modified_base 6: mod_base = OTHER; note = thymine
  modified_base 11: mod_base = OTHER; note = thymine
  modified_base 17: mod_base = OTHER; note = thymine
  misc_feature 1..18: note = antisense_mTOR of set 4
  source 1..18: mol_type = other RNA
gactgtggcatccacctg

SEQ ID NO: 8 - RNA, 18 nt, synthetic construct
  modified_base 2: mod_base = OTHER; note = thymine
  modified_base 6: mod_base = OTHER; note = thymine
  modified_base 14: mod_base = OTHER; note = thymine
  misc_feature 1..18: note = antisense_STAT3 of set 4
  source 1..18: mol_type = other RNA
ctgactccgcggatggac

SEQ ID NO: 9 - RNA, 17 nt, synthetic construct
  modified_base 6: mod_base = OTHER; note = thymine
  modified_base 9: mod_base = OTHER; note = thymine
  modified_base 11: mod_base = OTHER; note = thymine
  modified_base 15: mod_base = OTHER; note = thymine
  misc_feature 1..17: note = antisense_mTOR of set 5
  source 1..17: mol_type = other RNA
caagctgctgtggctga

SEQ ID NO: 10 - RNA, 17 nt, synthetic construct
  modified_base 2..3: mod_base = OTHER; note = thymine
  modified_base 12: mod_base = OTHER; note = thymine
  modified_base 17: mod_base = OTHER; note = thymine
  misc_feature 1..17: note = antisense_STAT3 of set 5
  source 1..17: mol_type = other RNA
gttcgacgacatcgact

SEQ ID NO: 11 - RNA, 20 nt, synthetic construct
  modified_base 1: mod_base = OTHER; note = thymine
  modified_base 4: mod_base = OTHER; note = thymine
  modified_base 13: mod_base = OTHER; note = thymine
  modified_base 18: mod_base = OTHER; note = thymine
  misc_feature 1..20: note = antisense_mTOR of set 6
  source 1..20: mol_type = other RNA
tgctgggccgcatgcgctgc

SEQ ID NO: 12 - RNA, 20 nt, synthetic construct
  modified_base 12: mod_base = OTHER; note = thymine
  misc_feature 1..20: note = antisense_STAT3 of set 6
  source 1..20: mol_type = other RNA
acgacccggcgtcaccgacg

SEQ ID NO: 13 - RNA, 19 nt, synthetic construct
  modified_base 3: mod_base = OTHER; note = thymine
  modified_base 12: mod_base = OTHER; note = thymine
  modified_base 17: mod_base = OTHER; note = thymine
  misc_feature 1..19: note = antisense_mTOR of set 7
  source 1..19: mol_type = other RNA
gctgggccgcatgcgctgc

SEQ ID NO: 14 - RNA, 19 nt, synthetic construct
  modified_base 11: mod_base = OTHER; note = thymine
  misc_feature 1..19: note = antisense_STAT3 of set 7
  source 1..19: mol_type = other RNA
cgacccggcgtcaccgacg

SEQ ID NO: 15 - RNA, 18 nt, synthetic construct
  modified_base 2: mod_base = OTHER; note = thymine
  modified_base 11: mod_base = OTHER; note = thymine
  modified_base 16: mod_base = OTHER; note = thymine
  misc_feature 1..18: note = antisense_mTOR of set 8
  source 1..18: mol_type = other RNA
ctgggccgcatgcgctgc

SEQ ID NO: 16 - RNA, 18 nt, synthetic construct
  modified_base 10: mod_base = OTHER; note = thymine
  misc_feature 1..18: note = antisense_STAT3 of set 8
  source 1..18: mol_type = other RNA
gacccggcgtcaccgacg

SEQ ID NO: 17 - RNA, 17 nt, synthetic construct
  modified_base 1: mod_base = OTHER; note = thymine
  modified_base 10: mod_base = OTHER; note = thymine
  modified_base 15: mod_base = OTHER; note = thymine
  misc_feature 1..17: note = antisense_mTOR of set 9
  source 1..17: mol_type = other RNA
tgggccgcatgcgctgc

SEQ ID NO: 18 - RNA, 17 nt, synthetic construct
  modified_base 9: mod_base = OTHER; note = thymine
  misc_feature 1..17: note = antisense_STAT3 of set 9
  source 1..17: mol_type = other RNA
acccggcgtcaccgacg

SEQ ID NO: 19 - DNA, 276 bp, synthetic construct
  misc_feature 1..276: note = U7 promotor
  source 1..276: mol_type = other DNA
cctagagtcgacactagataacaacataggagctgtgattggctgttttcagccaatcagcactgactcatttgcatagcctttacaagcggtcacaaactcaagaaacgagcggttttaatagtcttttagaatattgtttatcgaaccgaataaggaactgtgctttgtgattcacatatcagtggaggggtgtggaaatggcaccttgatctcaccctcatcgaaagtggagttgatgtccttccctggctcgctacagacgcacttccgcaa

SEQ ID NO: 20 - RNA, 54 nt, synthetic construct
  modified_base 4: mod_base = OTHER; note = thymine
  modified_base 6: mod_base = OTHER; note = thymine
  modified_base 11: mod_base = OTHER; note = thymine
  modified_base 17: mod_base = OTHER; note = thymine
  modified_base 21..23: mod_base = OTHER; note = thymine
  modified_base 27: mod_base = OTHER; note = thymine
  modified_base 33: mod_base = OTHER; note = thymine
  modified_base 39: mod_base = OTHER; note = thymine
  modified_base 47: mod_base = OTHER; note = thymine
  modified_base 51: mod_base = OTHER; note = thymine
  modified_base 53..54: mod_base = OTHER; note = thymine
  misc_feature 1..54: note = TTGGATCCAA loop shRNA
  source 1..54: mol_type = other RNA
gactgtggcatccacctgcatttggatccaaatgcaggtaggcgcctcagtctt

SEQ ID NO: 21 - RNA, 54 nt, synthetic construct
  modified_base 4: mod_base = OTHER; note = thymine
  modified_base 6: mod_base = OTHER; note = thymine
  modified_base 11: mod_base = OTHER; note = thymine
  modified_base 17: mod_base = OTHER; note = thymine
  modified_base 21..23: mod_base = OTHER; note = thymine
  modified_base 33: mod_base = OTHER; note = thymine
  modified_base 39: mod_base = OTHER; note = thymine
  modified_base 47: mod_base = OTHER; note = thymine
  modified_base 51: mod_base = OTHER; note = thymine
  modified_base 53..54: mod_base = OTHER; note = thymine
  misc_feature 1..54: note = TTCAAGAGAG loop shRNA
  source 1..54: mol_type = other RNA
gactgtggcatccacctgcatttcaagagagatgcaggtaggcgcctcagtctt

SEQ ID NO: 22 - RNA, 21 nt, synthetic construct
  modified_base 4: mod_base = OTHER; note = thymine
  modified_base 6: mod_base = OTHER; note = thymine
  modified_base 11: mod_base = OTHER; note = thymine
  modified_base 17: mod_base = OTHER; note = thymine
  modified_base 21: mod_base = OTHER; note = thymine
  misc_feature 1..21: note = antisense_mTOR
  source 1..21: mol_type = other RNA
gactgtggcatccacctgcat

SEQ ID NO: 23 - RNA, 21 nt, synthetic construct
  modified_base 2: mod_base = OTHER; note = thymine
  modified_base 8: mod_base = OTHER; note = thymine
  modified_base 16: mod_base = OTHER; note = thymine
  modified_base 20: mod_base = OTHER; note = thymine
  misc_feature 1..21: note = antisense_STAT3
  source 1..21: mol_type = other RNA
atgcaggtaggcgcctcagtc

SEQ ID NO: 24 - RNA, 23 nt, synthetic construct
  modified_base 21: mod_base = OTHER; note = thymine
  modified_base 23: mod_base = OTHER; note = thymine
  misc_feature 1..23: note = mTOR siRNA_sense strand
  source 1..23: mol_type = other RNA
gtggaaacaggacccatgadtdt

SEQ ID NO: 25 - RNA, 23 nt, synthetic construct
  misc_feature 1..23: note = STAT3 siRNA_sense strand
  source 1..23: mol_type = other RNA
  modified_base 21: mod_base = OTHER; note = thymine
  modified_base 23: mod_base = OTHER; note = thymine
tcatgggtcctgtttccacdtdt